European Patent Application EP 4 756 031 A1, published June 10, 2026. Title: Novel promoter and uses thereof. Applicant: CJ CheilJedang Corporation. Application KR. The sequence listing filed with the application follows.

SEQUENCE LISTING (28 sequences)

SEQ ID NO: 1 - DNA, 318 bp, synthetic construct
  source 1..318: mol_type = other DNA
agaaacatcccagcgctactaatagggagcgttgaccttccttccacggaccggtaatcggagtgcctaaaaccgcatgcggcttaggctccaagataggttctgcgcggccgggtaatgcatcttctttagcaacaagttgaggggtaggtgcaaataagaacgacatagaaatcgtctcctttctgtttttaatcaacatacaccaccacctaaaaattccccgaccagcaagttcacagtattcgggcacaatatcgttgacaaaatattgtttcggaatataatgggatacgtacccaacgaaaggaaacactc

SEQ ID NO: 2 - DNA, 318 bp, synthetic construct
  source 1..318: mol_type = other DNA
agaaacatcccagcgctactaatagggagcgttgaccttccttccacggaccggtaatcggagtgcctaaaaccgcatgcggcttaggctccaagataggttctgcgcggccgggtaatgcatcttctttagcaacaagttgaggggtaggtgcaaataagaacgacatagaaatcgtctcctttctgtttttaatcaacatacaccaccacctaaaaattccccgaccagcaagttcacagtattcgggcacaatatcgttgacaaaatattgttttgtggtataatgggatacgtacccaacgaaaggaaacactc

SEQ ID NO: 3 - DNA, 318 bp, synthetic construct
  source 1..318: mol_type = other DNA
agaaacatcccagcgctactaatagggagcgttgaccttccttccacggaccggtaatcggagtgcctaaaaccgcatgcggcttaggctccaagataggttctgcgcggccgggtaatgcatcttctttagcaacaagttgaggggtaggtgcaaataagaacgacatagaaatcgtctcctttctgtttttaatcaacatacaccaccacctaaaaattccccgaccagcaagttcacagtattcgggcacaatatcgttgccaaaatattgttttgtggtatcatgggatacgtacccaacgaaaggaaacactc

SEQ ID NO: 4 - DNA, 318 bp, synthetic construct
  source 1..318: mol_type = other DNA
agaaacatcccagcgctactaatagggagcgttgaccttccttccacggaccggtaatcggagtgcctaaaaccgcatgcggcttaggctccaagataggttctgcgcggccgggtaatgcatcttctttagcaacaagttgaggggtaggtgcaaataagaacgacatagaaatcgtctcctttctgtttttaatcaacatacaccaccacctaaaaattccccgaccagcaagttcacagtattcgggcacaatatcgttgccaaaatattgtttcggaatatcatgggatacgtacccaacgaaaggaaacactc

SEQ ID NO: 5 - DNA, 44 bp, synthetic construct
  source 1..44: mol_type = other DNA
ccgctctagaactagtggatcccccagaaacatcccagcgctac

SEQ ID NO: 6 - DNA, 39 bp, synthetic construct
  source 1..39: mol_type = other DNA
gatatcgaattcctgcagcccttatttgtagagctcatc

SEQ ID NO: 7 - DNA, 25 bp, synthetic construct
  source 1..25: mol_type = other DNA
attggagctccaccgcggtggcggc

SEQ ID NO: 8 - DNA, 24 bp, synthetic construct
  source 1..24: mol_type = other DNA
ccagtgaaaagttcttctccttta

SEQ ID NO: 9 - DNA, 40 bp, synthetic construct
  source 1..40: mol_type = other DNA
gaaaaattttttatcttatcagaaacatcccagcgctact

SEQ ID NO: 10 - DNA, 40 bp, synthetic construct
  source 1..40: mol_type = other DNA
agttcttctcctttactcatgagtgtttcctttcgttggg

SEQ ID NO: 11 - DNA, 40 bp, synthetic construct
  source 1..40: mol_type = other DNA
tattggaggagatcaaaacaatgagtaaaggagaagaact

SEQ ID NO: 12 - DNA, 40 bp, synthetic construct
  source 1..40: mol_type = other DNA
aggcgggctgccccggggacttatttgtagagctcatcca

SEQ ID NO: 13 - DNA, 20 bp, synthetic construct
  source 1..20: mol_type = other DNA
gtccccggggcagcccgcct

SEQ ID NO: 14 - DNA, 20 bp, synthetic construct
  source 1..20: mol_type = other DNA
gataagataaaaaatttttc

SEQ ID NO: 15 - DNA, 40 bp, synthetic construct
  source 1..40: mol_type = other DNA
gaaaaattttttatcttatcattttacatttttagaaatg

SEQ ID NO: 16 - DNA, 40 bp, synthetic construct
  source 1..40: mol_type = other DNA
agttcttctcctttactcattgcatccacctcactacatt

SEQ ID NO: 17 - DNA, 40 bp, synthetic construct
  source 1..40: mol_type = other DNA
aatgtagtgaggtggatgcaatgagtaaaggagaagaact

SEQ ID NO: 18 - protein, 476 aa, Lactobacillus delbrueckii
MTEHYLNYVNGEWRDSADAIEIFEPATGKSLGTVPAMSHEDVDYVMNSAKKALPAWRALSYVERAAYLQKAADILYRDAEKIGSTLSKEIAKGLKSSIGEVTRTAEIVEYTAKVGVTLDGEVMEGGNFEAASKNKLAVVRREPVGLVLAISPFNYPVNLAGSKIAPALMGGNVVAFKPPTQGSISGLLLAKAFAEAGLPAGVFNTITGRGRVIGDYIVEHPAVNFINFTGSSAVGKNIGKLAGMRPIMLELGGKDAAIVLEDADLDLTAKNIVAGAFGYSGQRCTAVKRVLVMDSVADELVEKVTALAKDLTVGIPEEDADITPLIDTKSADYVQGLIEEAAEKGAKPLFDFKREGNLIYPMVMDQVTTDMRLAWEEPFGPVLPFIRVKSADEAVMIANESEYGLQSSVFSRNFEKAFAIAGKLEVGTVHINNKTQRGPDNFPFLGVKSSGAGVQGVKYSIQAMTRVKSVVFNIED

SEQ ID NO: 19 - DNA, 1431 bp, Lactobacillus delbrueckii
  source 1..1431: mol_type = genomic DNA
ttgacagaacactatttaaactatgtcaatggcgaatggcgggactccgctgacgcgattgaaattttcgaaccagcaactggcaagtccctgggtactgtacctgccatgtcccacgaagacgtggactacgtaatgaacagcgccaaaaaggcccttccagcctggcgggccctctcatacgttgaacgggccgcatacttgcaaaaggcagcggacatcctttaccgagatgctgaaaagatcggttctaccttgtccaaggaaatcgccaagggcctcaagtcctctatcggcgaagtaacccggacggcggaaatcgttgaatacacggccaaggtcggcgtaactttggacggggaagtcatggagggcggcaactttgaagcggcaagcaagaacaagttggctgttgtccgccgggaaccagtcggcctggttttggcaatttcacccttcaactacccggttaacctggccggctcaaagatcgcgcctgctttgatgggcgggaacgtggtggccttcaagccgccgacacaagggtcaatctccggtctgcttttggccaaggccttcgccgaagctggcctgccagccggcgtcttcaacaccattaccggccggggtcgggttatcggcgactacatcgttgaacacccggcagtcaacttcatcaacttcaccggttccagtgctgtcggcaagaacatcggcaaactggccgggatgcggccgattatgctggaacttggcggcaaggacgcggccatcgtcttggaagacgctgacttggacctgacggccaagaacatcgttgccggcgcctttggctactccggccagcgttgtaccgccgttaagcgggttctggtcatggacagcgtggctgacgaattggttgaaaaggtgactgctttggccaaggatttgacggtcgggataccagaagaggatgccgacatcactcctttgatcgacactaagtctgccgactacgtacaaggcttaattgaagaagccgcagaaaagggcgctaagcctttgtttgacttcaagcgcgaaggcaacctgatctacccaatggtcatggaccaagtgacgactgacatgcgcctggcctgggaagaaccatttggaccagtattgccattcatccgcgtcaagtcagctgacgaagctgtcatgattgccaatgaatcagaatacggccttcaaagctccgtcttctcacggaactttgaaaaagcctttgccattgcaggaaaattggaagtgggcacggtccacatcaacaacaagacccaaagaggtccggacaacttcccattcctgggcgtaaagagctcaggggcaggcgtacagggggtcaagtactccattcaagccatgacccgggtcaagtccgttgtcttcaacatcgaagactaa

SEQ ID NO: 20 - DNA, 40 bp, synthetic construct
  source 1..40: mol_type = other DNA
gcggccgctctagaactagtgagaaacatcccagcgctac

SEQ ID NO: 21 - DNA, 39 bp, synthetic construct
  source 1..39: mol_type = other DNA
tttaaatagtgttctgtcatgagtgtttcctttcgttgg

SEQ ID NO: 22 - DNA, 39 bp, synthetic construct
  source 1..39: mol_type = other DNA
ccaacgaaaggaaacactcatgacagaacactatttaaa

SEQ ID NO: 23 - DNA, 40 bp, synthetic construct
  source 1..40: mol_type = other DNA
ccccctcgaggtcgattagtcttcgatgttgaagacaacg

SEQ ID NO: 24 - DNA, 1104 bp, Corynebacterium glutamicum
  source 1..1104: mol_type = genomic DNA
atgacgtcattagagttcacagtaacccgtaccgaaaatccgacgtcacccgatcgtctgaaggaaattcttgccgcaccgaagttcggtaagtacttcaccgaccacatggtgaccattgactggaacgagtcggaaggctggcacaacgcccaattagtgccatacgcgccgattcctatggatcctgccaccaccgtattccactacggacaggcaatttttgagggaattaaggcctaccgccattcggacgaaaccatcaagactttccgtcctgatgaaaacgccgagcgtatgcagcgttcagcagctcgaatggcaatgccacagttgccaaccgaggactttattaaagcacttgaactgctggtagacgcggatcaggattgggttcctgagtacggcggggaagcttccctctacctgcgcccattcatgatctccaccgaaattggcttgggtgtcagcccagctgatgcctacaagttcctggtcatcgcatccccagtcggcgcttacttcaccggtggaatcaagcctgtttccgtctggctgagcgaagattacgtccgcgctgcacccggcggaactggtgacgccaaatttgctggcaactacgcggcttctttgcttgcccagtcccaggctgcggaaaagggctgtgaccaggtcgtatggttggatgccatcgagcacaagtacatcgaagaaatgggtggcatgaaccttgggttcatctaccgcaacggcgaccacgtcaagctagtcacccctgaactttccggctcactacttccaggcatcactcgcaagtcacttctacaagtagcacgcgacttgggctacgaagtagaagagcgaaagatcaccaccaccgagtgggaagaagacgcaaagtctggcgccatgaccgaggcatttgcttgcggtactgcagctgttatcacccctgttggcaccgtgaaatcagctcacggcaccttcgaagtgaacaacaatgaagtcggagaaatcacgatgaagcttcgtgaaaccctcaccggaattcagcaaggaaacgttgaagaccaaaacggatggctttacccactggttggctaa

SEQ ID NO: 25 - DNA, 34 bp, synthetic construct
  source 1..34: mol_type = other DNA
ctgcaggaattcgatagaaacatcccagcgctac

SEQ ID NO: 26 - DNA, 35 bp, synthetic construct
  source 1..35: mol_type = other DNA
tgaactctaatgacgtcatgagtgtttcctttcgt

SEQ ID NO: 27 - DNA, 35 bp, synthetic construct
  source 1..35: mol_type = other DNA
aacgaaaggaaacactcatgacgtcattagagttc

SEQ ID NO: 28 - DNA, 38 bp, synthetic construct
  source 1..38: mol_type = other DNA
ccccctcgaggtcgattagccaaccagtgggtaaagcc